European Patent Application EP 4 219 707 A1, published August 2, 2023. Title: METHOD FOR PREPARING EFFECTOR CELLS WITH DESIRED SPECIFICITY. Applicant: Kyoto University NATIONAL UNIVERSITY CORPORATION SHIGA UNIVERSITY OF MEDICAL SCIENCE. The sequence listing filed with the application follows.

SEQUENCE LISTING (16 sequences)

SEQ ID NO: 1 - DNA, 24 bp, Artificial Sequence
  Synthetic Sequence
caccgaggttagtctgactgtgtg

SEQ ID NO: 2 - DNA, 24 bp, Artificial Sequence
  Synthetic Sequence
aaaccacacagtcagactaacctc

SEQ ID NO: 3 - DNA, 24 bp, Artificial Sequence
  Synthetic Sequence
caccctgccgctgcccagtggttg

SEQ ID NO: 4 - DNA, 24 bp, Artificial Sequence
  Synthetic Sequence
aaaccaaccactgggcagcggcag

SEQ ID NO: 5 - DNA, 22 bp, Artificial Sequence
  Synthetic Sequence
acggctgaaatctccctaaccc

SEQ ID NO: 6 - DNA, 41 bp, Artificial Sequence
  Synthetic Sequence
atacgaagttatagctagtcttccgtgatggcctcacacca

SEQ ID NO: 7 - DNA, 18 bp, Artificial Sequence
  Synthetic Sequence
gtccagacccacgtcacc

SEQ ID NO: 8 - DNA, 20 bp, Artificial Sequence
  Synthetic Sequence
ggggaccgaggggctggaag

SEQ ID NO: 9 - DNA, 21 bp, Artificial Sequence
  Synthetic Sequence
cctcctgtcataaggtgccat

SEQ ID NO: 10 - DNA, 21 bp, Artificial Sequence
  Synthetic Sequence
ccactttgctgtcttggcctt

SEQ ID NO: 11 - DNA, 22 bp, Artificial Sequence
  Synthetic Sequence
agccaaaatctggtacacaagg

SEQ ID NO: 12 - DNA, 21 bp, Artificial Sequence
  Synthetic Sequence
ctgagcactacacgcgaagca

SEQ ID NO: 13 - DNA, 18 bp, Artificial Sequence
  Synthetic Sequence
tgtaaaacgacggccagt

SEQ ID NO: 14 - DNA, 21 bp, Artificial Sequence
  Synthetic Sequence
caggaaacagctatgaccatg

SEQ ID NO: 15 - DNA, 23 bp, Artificial Sequence
  Synthetic Sequence
gcatcgtacgcgtacgtgtttgg

SEQ ID NO: 16 - DNA, 55 bp, Artificial Sequence
  Synthetic Sequence
cagcttctacatctgcagtgctagagcagggacgggtggggccaacgtcctgact